European Patent Application EP 4 238 581 A1, published September 6, 2023. Title: Targeted delivery of oligonucleotides into eukaryotic cells using hybrid maltose/cyclodextrin polyplexes. Applicant: Technische Universität Dresden Leibniz-Institut für Polymerforschung Dresden e. V. The sequence listing filed with the application follows.

SEQUENCE LISTING (13 sequences)

SEQ ID NO: 1 - protein, 464 aa, Mus musculus
METDTLLLWVLLLWVPGSTGDAAQPARRARRTKLGTELGSQVKLQESGGGLVQPGGSLKLSCVASGFTFSSYTMSWVRRTPEKRLEWVAYIHNGGGHTYYPDTIKGRFTISRDNAKNTLFLEMSSLKSEDTAMYYCTRRMYYGNSHWYFDVWGAGTSVTVSSAKTTPPSVYGGGGSGGGGSGGGGSTNSDIVMTQSPSSLSASLGDRVTINCRTSQDISNYLNWYQLTPDGTVKLLIYYTLKLNSGVPSRFSGSGSGTDYSLTINNLEKEDFATYFCQQSKTLPWTFGGGTKLEIKRADAAPTVSGPKLSSKLKVTVNGTAYDVDVDVDKSHENPMGTILFGGGTGGAPAPAAGGAGAGKAGEGEIPAPLAGTVSKILVKEGDTVKAGQTVLVLEAMKMETEINAPTDGKVEKVLVKERDAVQGGQGLIKIGDLELIEGSSGPEQKLISEEDLNSAVDHHHHHH

SEQ ID NO: 2 - protein, 126 aa, Artificial sequence
  transcarboxylase fragment
MKLKVTVNGTAYDVDVDVDKSHENPMGTILFGGGTGGAPAPAAGGAGAGKAGEGEIPAPLAGTVSKILVKEGDTVKAGQTVLVLEAMKMETEINAPTDGKVEKVLVKERDAVQGGQGLIKIGDLEL

SEQ ID NO: 3 - protein, 68 aa, Artificial sequence
  BCCP domain
VLRSPMPGVVVAVSVKPGDAVAEGQEICVIEAMKMQNSMTAGKTGTVKSVHCQAGDTVGEGDLLVELE

SEQ ID NO: 4 - protein, 13 aa, Artificial sequence
  Synthetic peptide
  VARIANT (2)..(2): Xaa is any amino acid
  VARIANT (3)..(3): Xaa is any amino acid except Leu, Val, Ile, Trp, Phe or Tyr
LXXIFEAQKIEWR

SEQ ID NO: 5 - protein, 15 aa, Artificial sequence
  Synthetic peptide
GLNDIFEAQKIEWHE

SEQ ID NO: 6 - protein, 15 aa, Artificial sequence
  Synthetic peptide
ALNDIFEAQKIEWHA

SEQ ID NO: 7 - protein, 23 aa, Artificial sequence
  Synthetic peptide
MAGGLNDIFEAQKIEWHEDTGGS

SEQ ID NO: 8 - protein, 23 aa, Artificial sequence
  Synthetic peptide
MSGLNDIFEAQKIEWHEGAPSSR

SEQ ID NO: 9 - protein, 15 aa, Artificial sequence
  Synbthetic peptide
LHHILDAQKMVWNHR

SEQ ID NO: 10 - protein, 10 aa, Artificial sequence
  Synthetic peptide
EQKLISEEDL

SEQ ID NO: 11 - protein, 392 aa, Homo sapiens
MEEPQSDPSVEPPLSQETFSDLWKLLPENNVLSPLPSQAMDDLMLSPDDIEQWFTEDPGPDEAPRMPEAAPRVAPAPAAPTPAAPAPAPSWPLSSSVPSQKTYQGSYGFRLGFLHSGTAKSVTCTYSPALNKMFCQLAKTCPVQLWVDSTPPPGTRVRAMAIYKQSQHMTEVVRRCPHHERCSDSDGLAPPQHLIRVEGNLRVEYLDDRNTFRHSVVVPYEPPEVGSDCTTIHYNYMCNSSCMGGMNRRPILTIITLEDSSGNLLGRNSFEVRVCACPGRDRRTEEENLRKKGEPHHELPPGSTKRALPNTSSSPQPKKKPLDGEYFTLQIRGRERFEMFRELNEALELKDAQAGKEPGGSRAHSSHLKSKKGQSTSRHKKLMFKTEGPDSD

SEQ ID NO: 12 - protein, 328 aa, Artificial sequence
  Rekombinant polypeptide
METDTLLLWVLLLWVPGSTGDAAQPARRARRTKLGTELGSEVQLLESGGGLVQPGGSLRLSCVASGFTFSSYTMSWVRQAPGKGLEWVSYIHNGGGHTYYADSVKGRFTISRDNSKNTLYLQMNSLRAEDTAVYYCTRRMYYGNSHWYFDVWGAGTRVTITSAKTTPPSVYGGGGSGGGGSGGGGSTNSDIQMTQSPSSLSASVGDRVTITCRTSQSISNYLNWYQQKPGKAPKLLIYYTLKLNSGVPSRFSGSGSGTDFTLTISSLQPEDFATYYCQQSKTLPWTFGGGTKLEIKRADAAPTVSGPEQKLISEEDLNSAVDHHHHHH

SEQ ID NO: 13 - protein, 326 aa, Artificial sequence
  Recombinant polypeptide
MRVPAQLLGLLLLWFPGVRCGDGSAAQPARRARRTKLHMQVKLQQSGGGLVKPGASLKLSCVTSGFTFRKFGMSWVRQTSDKRLEWVASISTGGYNTYYSDNVKGRFTISRENAKNTLYLQMSSLKSEDTALYYCTRGYSPYSYAMDYWGQGTTVTVSSSGGGSGGGGSGGGGSDIELTQSPASLSVATGEKATIRCMTSTDIDDDMNWYQQKPGEPPKFLISEGNTLRPGVPSRFSSSGTGTDFVFTIENTLSEDVGDYYCLQSWNVPLTFGDGTKLEITDPLQCGGILQISSTVAAARGGPEQKLISEEDLNSAVDGGHHHHHH